European Patent Application EP 4 427 809 A2, published September 11, 2024. Title: ALTERING GENE EXPRESSION IN CART CELLS AND USES THEREOF. Applicant: The Trustees of the University of Pennsylvania. Application EP. The sequence listing filed with the application follows.

SEQUENCE LISTING (68 sequences)

SEQ ID NO: 1 - DNA, 20 bp, synthetic construct
  misc_feature 1..20: note = Synthetic sequence
  source 1..20: mol_type = other DNA
tgtgctagacatgaggtcta

SEQ ID NO: 2 - DNA, 20 bp, synthetic construct
  misc_feature 1..20: note = Synthetic sequence
  source 1..20: mol_type = other DNA
gcagtatctggagtcattga

SEQ ID NO: 3 - DNA, 20 bp, synthetic construct
  misc_feature 1..20: note = Synthetic sequence
  source 1..20: mol_type = other DNA
cgcgagcacagctaaggcca

SEQ ID NO: 4 - DNA, 20 bp, synthetic construct
  misc_feature 1..20: note = Synthetic sequence
  source 1..20: mol_type = other DNA
ggcgccctggccagtcgtct

SEQ ID NO: 5 - DNA, 20 bp, synthetic construct
  misc_feature 1..20: note = Synthetic sequence
  source 1..20: mol_type = other DNA
gagggtccagatgcccagca

SEQ ID NO: 6 - DNA, 24 bp, synthetic construct
  misc_feature 1..24: note = Synthetic sequence
  source 1..24: mol_type = other DNA
tcatgtcctaaccctgatcctctt

SEQ ID NO: 7 - DNA, 23 bp, synthetic construct
  misc_feature 1..23: note = Synthetic sequence
  source 1..23: mol_type = other DNA
ttggacttttcccagctgacaga

SEQ ID NO: 8 - DNA, 24 bp, synthetic construct
  misc_feature 1..24: note = Synthetic sequence
  source 1..24: mol_type = other DNA
taccaggaccagacagctcttaga

SEQ ID NO: 9 - DNA, 24 bp, synthetic construct
  misc_feature 1..24: note = Synthetic sequence
  source 1..24: mol_type = other DNA
tctcacctaatctcctccaggcat

SEQ ID NO: 10 - RNA, 54 nt, synthetic construct
  misc_feature 1..54: note = Synthetic sequence
  source 1..54: mol_type = other RNA
rargrgrargrgrartrtrcrgrgrararcrcrcrarartrcrarcrtrgrarc

SEQ ID NO: 11 - DNA, 48 bp, synthetic construct
  misc_feature 1..48: note = Synthetic sequence
  source 1..48: mol_type = other DNA
  misc_RNA 8
  misc_RNA 14
  misc_RNA 16
  misc_RNA 24
  misc_RNA 26
  misc_RNA 38
  misc_RNA 44
rcrargrtrgrartrtrgrgrgrtrtrcrcrgrarartrcrcrtrcct

SEQ ID NO: 12 - RNA, 54 nt, synthetic construct
  misc_feature 1..54: note = Synthetic sequence
  source 1..54: mol_type = other RNA
rarcrcrtrcrcrtrtrcrcrcrartrtrcrarcrcrcrarcrcrargrcrtrc

SEQ ID NO: 13 - DNA, 48 bp, synthetic construct
  misc_feature 1..48: note = Synthetic sequence
  source 1..48: mol_type = other DNA
  misc_RNA 6
  misc_RNA 12
  misc_RNA 20
  misc_RNA 28
rgrcrtrgrgrtrgrgrgrtrgrarartrgrgrgrarargrgrarggt

SEQ ID NO: 14 - DNA, 122 bp, synthetic construct
  misc_feature 1..122: note = Synthetic sequence; Figure 1B
  source 1..122: mol_type = other DNA
ttaatacgactcactataggcaccaaagctgcccttaccgttttagagctagaaatagcaagttaaaataaggctagtccgttatcaacttgaaaaagtggcaccgagtcggtgcttttttt

SEQ ID NO: 15 - DNA, 23 bp, synthetic construct
  misc_feature 1..23: note = Synthetic sequence; Figure 1C, Figure 3B, & Figure 21
  source 1..23: mol_type = other DNA
tgtgctagacatgaggtctatgg

SEQ ID NO: 16 - DNA, 23 bp, synthetic construct
  misc_feature 1..23: note = Synthetic sequence; Figure 1C, Figure 3B, & Figure 21
  source 1..23: mol_type = other DNA
ccctcaatgactccagatactgc

SEQ ID NO: 17 - DNA, 38 bp, synthetic construct
  misc_feature 1..38: note = Synthetic sequence; Figure 79B
  source 1..38: mol_type = other DNA
tgggctggcggccaggatggttcttggtaggtaggtgg

SEQ ID NO: 18 - DNA, 38 bp, synthetic construct
  misc_feature 1..38: note = Synthetic sequence; Figure 79B
  source 1..38: mol_type = other DNA
tgggctggcggccaggatggttcttaggggtaggtggg

SEQ ID NO: 19 - DNA, 67 bp, synthetic construct
  misc_feature 1..67: note = Synthetic sequence; Figure 3D & Figure 53A
  source 1..67: mol_type = other DNA
tatatcacagacaaaactgtgctagacatgaggtctatggacttcaagagcaacagtgctgtggcct

SEQ ID NO: 20 - DNA, 66 bp, synthetic construct
  misc_feature 1..66: note = Synthetic sequence; Figure 3D & Figure 53A
  source 1..66: mol_type = other DNA
tatatcacagacaaaactgtgctagacatgagtctatggacttcaagagcaacagtgctgtggcct

SEQ ID NO: 21 - DNA, 65 bp, synthetic construct
  misc_feature 1..65: note = Synthetic sequence; Figure 3D & Figure 53A
  source 1..65: mol_type = other DNA
tatatcacagacaaaactgtgctagacatggtctatggacttcaagagcaacagtgctgtggcct

SEQ ID NO: 22 - DNA, 66 bp, synthetic construct; identical to SEQ ID NO: 20
  misc_feature 1..66: note = Synthetic sequence; Figure 3D & Figure 53A
  source 1..66: mol_type = other DNA

SEQ ID NO: 23 - DNA, 64 bp, synthetic construct
  misc_feature 1..64: note = Synthetic sequence; Figure 3D & Figure 53A
  source 1..64: mol_type = other DNA
tatatcacagacaaaactgtgctagacatgtctatggacttcaagagcaacagtgctgtggcct

SEQ ID NO: 24 - DNA, 66 bp, synthetic construct
  misc_feature 1..66: note = Synthetic sequence; Figure 3D & Figure 53A
  source 1..66: mol_type = other DNA
tatatcacagacaaaactgtgctagactgaggtctatggacttcaagagcaacagtgctgtggcct

SEQ ID NO: 25 - DNA, 64 bp, Artificial sequence
  misc_feature 1..64: note = Synthetic sequence; Figure 3D & Figure 53A
  source 1..64: mol_type = other DNA
tatatcacagacaaaactgtgctagtgaggtctatggacttcaagagcaacagtgctgtggcct

SEQ ID NO: 26 - DNA, 62 bp, synthetic construct
  misc_feature 1..62: note = Synthetic sequence; Figure 3D & Figure 53A
  source 1..62: mol_type = other DNA
tatatcacagacaaaactgtgcttgaggtctatggacttcaagagcaacagtgctgtggcct

SEQ ID NO: 27 - DNA, 67 bp, synthetic construct
  misc_feature 1..67: note = Synthetic sequence; Figure 3D & Figure 53A
  source 1..67: mol_type = other DNA
tatatcacagacaaaactgtgctagacatgaggttctatggacttcaagagcaacagtgctgtggcc

SEQ ID NO: 28 - DNA, 67 bp, synthetic construct
  misc_feature 1..67: note = Synthetic sequence; Figure 3D & Figure 53A
  source 1..67: mol_type = other DNA
tatatcacagacaaaactgtgctagacatgagggtctatggacttcaagagcaacagtgctgtggcc

SEQ ID NO: 29 - DNA, 67 bp, synthetic construct
  misc_feature 1..67: note = Synthetic sequence; Figure 3D & Figure 53A
  source 1..67: mol_type = other DNA
agcagcccgccctcaatgactccagatactgcctgagcagccgcctgagggtctcggccaccttctg

SEQ ID NO: 30 - DNA, 66 bp, synthetic construct
  misc_feature 1..66: note = Synthetic sequence; Figure 3D & Figure 53A
  source 1..66: mol_type = other DNA
agcagcccgccctcatgactccagatactgcctgagcagccgcctgagggtctcggccaccttctg

SEQ ID NO: 31 - DNA, 66 bp, synthetic construct
  misc_feature 1..66: note = Synthetic sequence; Figure 3D & Figure 53A
  source 1..66: mol_type = other DNA
agcagcccgcctcaatgactccagatactgcctgagcagccgcctgagggtctcggccaccttctg

SEQ ID NO: 32 - DNA, 66 bp, synthetic construct
  misc_feature 1..66: note = Synthetic sequence; Figure 3D & Figure 53A
  source 1..66: mol_type = other DNA
agcagcccgccctcaatgactcagatactgcctgagcagccgcctgagggtctcggccaccttctg

SEQ ID NO: 33 - DNA, 65 bp, synthetic construct
  misc_feature 1..65: note = Synthetic sequence; Figure 3D & Figure 53A
  source 1..65: mol_type = other DNA
agcagcccgccctcaatgactagatactgcctgagcagccgcctgagggtctcggccaccttctg

SEQ ID NO: 34 - DNA, 62 bp, synthetic construct
  misc_feature 1..62: note = Synthetic sequence; Figure 3D & Figure 53A
  source 1..62: mol_type = other DNA
agcagcccgcccgactccagatactgcctgagcagccgcctgagggtctcggccaccttctg

SEQ ID NO: 35 - DNA, 67 bp, synthetic construct
  misc_feature 1..67: note = Synthetic sequence; Figure 3D & Figure 53A
  source 1..67: mol_type = other DNA
agcagcccgccctcaaatgactccagatactgcctgagcagccgcctgagggtctcggccaccttct

SEQ ID NO: 36 - DNA, 67 bp, synthetic construct
  misc_feature 1..67: note = Synthetic sequence; Figure 3D & Figure 53A
  source 1..67: mol_type = other DNA
agcagcccgccctcaatgactcccagatactgcctgagcagccgcctgagggtctcggccaccttct

SEQ ID NO: 37 - DNA, 67 bp, synthetic construct; identical to SEQ ID NO: 29
  misc_feature 1..67: note = Synthetic sequence; Figure 3D & Figure 53A
  source 1..67: mol_type = other DNA

SEQ ID NO: 38 - DNA, 64 bp, synthetic construct
  misc_feature 1..64: note = Synthetic sequence; Figure 3D & Figure 53A
  source 1..64: mol_type = other DNA
agcagcccgccctcaatgacagatactgcctgagcagccgcctgagggtctcggccaccttctg

SEQ ID NO: 39 - DNA, 66 bp, synthetic construct; identical to SEQ ID NO: 32
  misc_feature 1..66: note = Synthetic sequence; Figure 3D & Figure 53A
  source 1..66: mol_type = other DNA

SEQ ID NO: 40 - DNA, 55 bp, synthetic construct
  misc_feature 1..55: note = Synthetic sequence; Figure 3D & Figure 53A
  source 1..55: mol_type = other DNA
agcagcccgccctcaactgcctgagcagccgcctgagggtctcggccaccttctg

SEQ ID NO: 41 - DNA, 62 bp, synthetic construct
  misc_feature 1..62: note = Synthetic sequence; Figure 3D & Figure 53A
  source 1..62: mol_type = other DNA
agcagcccgcctcatgactcagatactgctgagcagccgcctgagggtctcggccaccttct

SEQ ID NO: 42 - DNA, 46 bp, synthetic construct
  misc_feature 1..46: note = Synthetic sequence; Figure 3D & Figure 53A
  source 1..46: mol_type = other DNA
agcagccactgcgtgagcagccgcgtgagggtctcggccaccttct

SEQ ID NO: 43 - DNA, 67 bp, synthetic construct
  misc_feature 1..67: note = Synthetic sequence; Figure 3D & Figure 53A
  source 1..67: mol_type = other DNA
agcagcccgccctcaatgactccgagatactgcctgagcagccgcctgagggtctcggccaccttct

SEQ ID NO: 44 - DNA, 23 bp, synthetic construct
  misc_feature 1..23: note = Synthetic sequence; Figure 9A
  source 1..23: mol_type = other DNA
ccgtggccttagctgtgctcgcg

SEQ ID NO: 45 - DNA, 23 bp, synthetic construct
  misc_feature 1..23: note = Synthetic sequence; Figure 12A
  source 1..23: mol_type = other DNA
ccatgctgggcatctggaccctc

SEQ ID NO: 46 - DNA, 23 bp, synthetic construct
  misc_feature 1..23: note = Synthetic sequence; Figure 14A
  source 1..23: mol_type = other DNA
gggcggtgctacaactgggctgg

SEQ ID NO: 47 - DNA, 23 bp, synthetic construct
  misc_feature 1..23: note = Synthetic sequence; Figure 15A
  source 1..23: mol_type = other DNA
cataaagccatggcttgccttgg

SEQ ID NO: 48 - DNA, 64 bp, synthetic construct
  misc_feature 1..64: note = Synthetic sequence; Figure 15B
  source 1..64: mol_type = other DNA
aacaccgctcccataaagccatggcttgccttggatttcagcggcacaaggctcagctgaacct

SEQ ID NO: 49 - DNA, 59 bp, synthetic construct
  misc_feature 1..59: note = Synthetic sequence; Figure 15B
  source 1..59: mol_type = other DNA
aacaccgctcccataatggcttgccttggatttcagcggcacaaggctcagctgaacct

SEQ ID NO: 50 - DNA, 62 bp, synthetic construct
  misc_feature 1..62: note = Synthetic sequence; Figure 15B
  source 1..62: mol_type = other DNA
aacaccgctcccataaccatggcttgccttggatttcagcggcacaaggctcagctgaacct

SEQ ID NO: 51 - DNA, 62 bp, synthetic construct; identical to SEQ ID NO: 50
  misc_feature 1..62: note = Synthetic sequence; Figure 15B
  source 1..62: mol_type = other DNA

SEQ ID NO: 52 - DNA, 64 bp, synthetic construct
  misc_feature 1..64: note = Synthetic sequence; Figure 15B
  source 1..64: mol_type = other DNA
aacaccgctcccataaagtccatggcttgccttggatttcagcggcacaaggctcagctgaacc

SEQ ID NO: 53 - DNA, 63 bp, synthetic construct
  misc_feature 1..63: note = Synthetic sequence; Figure 15B
  source 1..63: mol_type = other DNA
aacaccgctcccataaaccatggcttgccttggatttcagcggcacaaggctcagctgaacct

SEQ ID NO: 54 - DNA, 50 bp, synthetic construct
  misc_feature 1..50: note = Synthetic sequence; Figure 15B
  source 1..50: mol_type = other DNA
aacaccgctcccataaagggatttcagcggcacaaggctcagctgaacct

SEQ ID NO: 55 - DNA, 59 bp, synthetic construct; identical to SEQ ID NO: 49
  misc_feature 1..59: note = Synthetic sequence; Figure 15B
  source 1..59: mol_type = other DNA

SEQ ID NO: 56 - DNA, 59 bp, synthetic construct; identical to SEQ ID NO: 49
  misc_feature 1..59: note = Synthetic sequence; Figure 15B
  source 1..59: mol_type = other DNA

SEQ ID NO: 57 - DNA, 63 bp, synthetic construct; identical to SEQ ID NO: 53
  misc_feature 1..63: note = Synthetic sequence; Figure 15B
  source 1..63: mol_type = other DNA

SEQ ID NO: 58 - DNA, 61 bp, synthetic construct
  misc_feature 1..61: note = Synthetic sequence; Figure 15B
  source 1..61: mol_type = other DNA
aacaccgctcccataccatggcttgccttggatttcagcggcacaaggctcagctgaacct

SEQ ID NO: 59 - DNA, 59 bp, synthetic construct; identical to SEQ ID NO: 49
  misc_feature 1..59: note = Synthetic sequence; Figure 15B
  source 1..59: mol_type = other DNA

SEQ ID NO: 60 - DNA, 64 bp, synthetic construct; identical to SEQ ID NO: 48
  misc_feature 1..64: note = Synthetic sequence; Figure 15B
  source 1..64: mol_type = other DNA

SEQ ID NO: 61 - DNA, 23 bp, synthetic construct
  misc_feature 1..23: note = Synthetic sequence; Figure 16
  source 1..23: mol_type = other DNA
ggacatcaagcctgctaacatgg

SEQ ID NO: 62 - DNA, 23 bp, synthetic construct
  misc_feature 1..23: note = Synthetic sequence; Figure 16
  source 1..23: mol_type = other DNA
catcaagcctgctaacatggagg

SEQ ID NO: 63 - DNA, 122 bp, synthetic construct
  misc_feature 1..122: note = Synthetic sequence; Figure 49
  misc_feature 19..39: note = n is a, c, g, or t
  source 1..122: mol_type = other DNA
taatacgactcactatagnnnnnnnnnnnnnnnnnnnnngttttagagctagaaatagcaagttaaaataaggctagtccgttatcaacttgaaaaagtggcaccgagtcggtgcttttttt

SEQ ID NO: 64 - DNA, 20 bp, synthetic construct
  misc_feature 1..20: note = Synthetic sequence; Figure 79A
  source 1..20: mol_type = other DNA
ggccaggatggttcttaggt

SEQ ID NO: 65 - DNA, 38 bp, synthetic construct
  misc_feature 1..38: note = Synthetic sequence; Figure 79B
  source 1..38: mol_type = other DNA
tgggctggcggccaggatggttcttaggtaggtggggt

SEQ ID NO: 66 - DNA, 34 bp, synthetic construct
  misc_feature 1..34: note = Synthetic sequence; Figure 79B
  source 1..34: mol_type = other DNA
tgggctggcggccaggatggtaggtaggtggggt

SEQ ID NO: 67 - DNA, 37 bp, synthetic construct
  misc_feature 1..37: note = Synthetic sequence; Figure 79B
  source 1..37: mol_type = other DNA
tgggctggcggccaggatggttttaggtaggtggggt

SEQ ID NO: 68 - DNA, 34 bp, synthetic construct; identical to SEQ ID NO: 66
  misc_feature 1..34: note = Synthetic sequence; Figure 79B
  source 1..34: mol_type = other DNA